European Patent Application EP 4 234 032 A2, published August 30, 2023. Title: INDUCTION MEDIUM AND METHODS FOR STEM CELL CULTURE AND THERAPY. Applicant: SanBio, Inc. Application EP EP23169770.7, filed September 24, 2015. The sequence listing filed with the application follows.

SEQUENCE LISTING (6 sequences)

SEQ ID NO: 1 - DNA, 21 bp, synthetic construct
  misc_feature 1..21: note = Cxcl9 Forward
  source 1..21: mol_type = other DNA
ctttcctggctactccatgtt

SEQ ID NO: 2 - DNA, 23 bp, synthetic construct
  misc_feature 1..23: note = Cxcl9 Reverse
  source 1..23: mol_type = other DNA
gttggtcactggctgatctataa

SEQ ID NO: 3 - DNA, 20 bp, synthetic construct
  misc_feature 1..20: note = Trail Forward
  source 1..20: mol_type = other DNA
cttcacagtgctcctgcagt

SEQ ID NO: 4 - DNA, 21 bp, synthetic construct
  misc_feature 1..21: note = Trail Reverse
  source 1..21: mol_type = other DNA
ttagccaactaaaaaggcccc

SEQ ID NO: 5 - DNA, 19 bp, synthetic construct
  misc_feature 1..19: note = 18SrRNA Forward
  source 1..19: mol_type = other DNA
gagggagcctgagaaacgg

SEQ ID NO: 6 - DNA, 20 bp, synthetic construct
  misc_feature 1..20: note = 18SrRNA Reverse
  source 1..20: mol_type = other DNA
gtcgggagtgggtaatttgc